European Patent Application EP 4 215 916 A1, published July 26, 2023. Title: Test zum Nachweis von Antikörpern gegen Leishmanien. Applicant: Philipps-Universität Marburg. The sequence listing filed with the application follows.

SEQUENCE LISTING (8 sequences)

SEQ ID NO: 1 - DNA, 22 bp, Artificial Sequence
  Forward Primer putative kinesin K39 Leishmania infantum
gagctcgcaaccgagtgggagg

SEQ ID NO: 2 - DNA, 17 bp, Artificial Sequence
  Reverse primer putative kinesin K39 Leishmania infantum
gctccgcagcgcgctcc

SEQ ID NO: 3 - DNA, 1117 bp, Artificial Sequence
  DNA Sequenz KLi8.3
gagctcgcaaccgagtgggaggacgcactccgcgagcgtgcgcttgcagagcgtgacgaagccgctgcagccgaacttgatgccgcagcctctacttcccaaaacgcacgtgaaagcgcctccgagcggctaaccagccttgagcagctgcttcgcgaatccgaggagcgcgctgcggagctggcgagtcagctggagtccactactgctgcgaagatgtcggcggagcaggaccgcgagaacacgagggccacgctagagcagcagcttcgtgactccgaggagcgcgctgcggagctggcgagccagctggaggccactgctgctgcgaagtcgtcggcggagcaggaccgcgagaacacgagggccgcgttggagcagctgcttcgcgaatccgaggagcgcgctgcggagctggcgagccagctggaggccactgctgctgcgaagatgtcggcggagcaggaccgcgagaacacgagggccgcgttggagcagcagcttcgtgactccgaggagcgcgctgcggagctggcgagtcagctggagtccactactgctgcgaagatgtcggcggagcaggaccgcgagaacacgagggccacgctagagcagcagcttcgtgactccgaggagcgcgctgcggagctggcgagtcagctggagtccactactgctgcgaagacgtcggcggagcaggaccgcgagaacacgagggccgcgttggagcagcagcttcgtgactccgaggagcgcgctgcggagctggcgagccagctggaggccactgctgctgcgaagtcgtcggcggagcaggaccgcgagaacacgagggccgcgttggagcagcagcttcgtgactccgaggagcgcgctgcggagctggcgagccagctggaggccactgctgctgcgaagtcgtcggcggagcaggaccgcgagaacacgagggccacgctagagcagcagcttcgtgactccgaggagcgcgctgcggagctggcgagtcagctggagtccactactgctgcgaagatgtcggcggagcaggaccgcgagaacacgagggccacgctagagcagcagcttcgtgactccgaggagcgcgctgcggagc

SEQ ID NO: 4 - protein, 326 aa, Artificial Sequence
  Aminosäuren-Repeat-Sequenz KLi8.3
LEQLLRESEERAAELASQLESTTAAKMSAEQDRENTRATLEQQLRDSEERAAELASQLEATAAAKSSAEQDRENTRAALEQLLRESEERAAELASQLEATAAAKMSAEQDRENTRAALEQQLRDSEERAAELASQLESTTAAKMSAEQDRENTRATLEQQLRDSEERAAELASQLESTTAAKTSAEQDRENTRAALEQQLRDSEERAAELASQLEATAAAKSSAEQDRENTRAALEQQLRDSEERAAELASQLEATAAAKSSAEQDRENTRATLEQQLRDSEERAAELASQLESTTAAKMSAEQDRENTRATLEQQLRDSEERAAE

SEQ ID NO: 5 - DNA, 36 bp, Artificial Sequence
  Forward Primer für DNA-Konstrukt pCR2.1/KLi8.3
gtacatatggagctcgcaaccgagtgggaggacgca

SEQ ID NO: 6 - DNA, 41 bp, Artificial Sequence
  Reverse primer für DNA-Konstrukt pCR2.1/KLi8.3
tacctcgagcagtgtgctggaattcgcccttactccgcagc

SEQ ID NO: 7 - DNA, 1182 bp, Artificial Sequence
  Nukleotidsequenz von rekombinantem 6xhis-KLi8.3 für his-KLi8.3-Fusionsprotein
atgggcagcagccatcatcatcatcatcacagcagcggcctggtgccgcgcggcagccatatggagctcgcaaccgagtgggaggacgcactccgcgagcgtgcgcttgcagagcgtgacgaagccgctgcagccgaacttgatgccgcagcctctacttcccaaaacgcacgtgaaagcgcctccgagcggctaaccagccttgagcagctgcttcgcgaatccgaggagcgcgctgcggagctggcgagtcagctggagtccactactgctgcgaagatgtcggcggagcaggaccgcgagaacacgagggccacgctagagcagcagcttcgtgactccgaggagcgcgctgcggagctggcgagccagctggaggccactgctgctgcgaagtcgtcggcggagcaggaccgcgagaacacgagggccgcgttggagcagctgcttcgcgaatccgaggagcgcgctgcggagctggcgagccagctggaggccactgctgctgcgaagatgtcggcggagcaggaccgcgagaacacgagggccgcgttggagcagcagcttcgtgactccgaggagcgcgctgcggagctggcgagtcagctggagtccactactgctgcgaagatgtcggcggagcaggaccgcgagaacacgagggccacgctagagcagcagcttcgtgactccgaggagcgcgctgcggagctggcgagtcagctggagtccactactgctgcgaagacgtcggcggagcaggaccgcgagaacacgagggccgcgttggagcagcagcttcgtgactccgaggagcgcgctgcggagctggcgagccagctggaggccactgctgctgcgaagtcgtcggcggagcaggaccgcgagaacacgagggccgcgttggagcagcagcttcgtgactccgaggagcgcgctgcggagctggcgagccagctggaggccactgctgctgcgaagtcgtcggcggagcaggaccgcgagaacacgagggccacgctagagcagcagcttcgtgactccgaggagcgcgctgcggagctggcgagtcagctggagtccactactgctgcgaagatgtcggcggagcaggaccgcgagaacacgagggccacgctagagcagcagcttcgtgactccgaggagcgcgctgcggagtaa

SEQ ID NO: 8 - protein, 393 aa, Artificial Sequence
  Aminosäuresequenz von rekombinantem 6xhis-rKLi8.3 für gereinigtes rKLi8.3-Protein
MGSSHHHHHHSSGLVPRGSHMELATEWEDALRERALAERDEAAAAELDAAASTSQNARESASERLTSLEQLLRESEERAAELASQLESTTAAKMSAEQDRENTRATLEQQLRDSEERAAELASQLEATAAAKSSAEQDRENTRAALEQLLRESEERAAELASQLEATAAAKMSAEQDRENTRAALEQQLRDSEERAAELASQLESTTAAKMSAEQDRENTRATLEQQLRDSEERAAELASQLESTTAAKTSAEQDRENTRAALEQQLRDSEERAAELASQLEATAAAKSSAEQDRENTRAALEQQLRDSEERAAELASQLEATAAAKSSAEQDRENTRATLEQQLRDSEERAAELASQLESTTAAKMSAEQDRENTRATLEQQLRDSEERAAE